European Patent Specification EP 4 384 602 B1, published March 25, 2026. Title: PLATELETS TRANSFECTED WITH SIRNA AND THE THERAPEUTIC USES THEREOF. Applicant: PLASFER SRL. The sequence listing filed with the application follows.

SEQUENCE LISTING (6 sequences)

SEQ ID NO: 1 - RNA, 21 nt, synthetic construct
  source 1..21: mol_type = other RNA
  modified_base 20..21: mod_base = OTHER; note = thymine
gttggagctgatggcgtagtt

SEQ ID NO: 2 - RNA, 21 nt, synthetic construct
  source 1..21: mol_type = other RNA
  modified_base 20..21: mod_base = OTHER; note = thymine
ctacgccatcagctccaactt

SEQ ID NO: 3 - DNA, 21 bp, Homo sapiens
  source 1..21: mol_type = genomic DNA
acttgtggtagttggagcaga

SEQ ID NO: 4 - DNA, 21 bp, Homo sapiens
  source 1..21: mol_type = genomic DNA
ttggatcatattcgtccacaa

SEQ ID NO: 5 - DNA, 23 bp, Homo sapiens
  source 1..23: mol_type = genomic DNA
gcttaatttgactcaacacggga

SEQ ID NO: 6 - DNA, 23 bp, Homo sapiens
  source 1..23: mol_type = genomic DNA
agctatcaatctgtcaatcctgt